European Patent Application EP 4 800 121 A1, published September 2, 2026. Title: RNA 변형의 모든 주변 서열을 포함하는 광범위한 RNA 변형 라이브러리 설계법 및 그 이용. Applicant: Seoul National University R&DB Foundation. Application KR. The sequence listing filed with the application follows.

SEQUENCE LISTING (5 sequences)

SEQ ID NO: 1 - RNA, 15 nt, synthetic construct
  source 1..15: mol_type = other RNA
cgacagatgagttcc

SEQ ID NO: 2 - RNA, 15 nt, synthetic construct
  source 1..15: mol_type = other RNA
ccttgatagacagtc

SEQ ID NO: 3 - DNA, 20 bp, synthetic construct
  source 1..20: mol_type = other DNA
tcatctgtcggactgtctat

SEQ ID NO: 4 - RNA, 30 nt, synthetic construct
  source 1..30: mol_type = other RNA
ggtacccgggcgaattccaagcttgatcgc

SEQ ID NO: 5 - RNA, 274 nt, synthetic construct
  source 1..274: mol_type = other RNA
gggcgagctcggtacccgggcgaattccaagcttgatcgcggagctctaggaagctcaaactttcctgatcctgcgggcaagctaaaccagttccggaagaacctgcgggagtcgcagcagctccgatgggacagtggctgggtgcagactgtgctccctttggttatggacacataactcctgggccagaggctaaaaccccaggacccctgctgtccttcccgcagcttcttcttggagtctgctataggctagcgaccgtcgatctggatc